European Patent Specification EP 3 512 943 B1, published April 12, 2023. Title: CRISP-SEQ, AN INTEGRATED METHOD FOR MASSIVELY PARALLEL SINGLE CELL RNA-SEQ AND CRISPR POOLED SCREENS. Applicant: Yeda Research and Development Co. Ltd. AMIT, Ido JAITIN, Diego LARA-ASTIASO, David WEINER, Assaf YOFE, Ido. The sequence listing filed with the application follows.

SEQUENCE LISTING (17 sequences)

SEQ ID NO: 1 - DNA, 64 bp, Artificial sequence
  Single strand DNA oligonucleotide
  misc_feature (36)..(43): n is a, c, g, or t
ctccctttgggccgcctccccgcgtcgacggatccnnnnnnnngacttacaaggcagctgtaga

SEQ ID NO: 2 - DNA, 20 bp, Artificial sequence
  UGI ligation adapter
  misc_feature (1)..(1): 5' Phosphate
  misc_feature (20)..(20): 3'  C3 spacer (blocker)
atgatcaagcgaccaccgag

SEQ ID NO: 3 - DNA, 20 bp, Artificial sequence
  Single strand DNA oligonucleotide
ctcggtggtcgcttgatcat

SEQ ID NO: 4 - DNA, 49 bp, Artificial sequence
  Single strand DNA oligonucleotide
  misc_feature (23)..(31): n is a, c, g, or t
ctacacgacgctcttccgatctnnnnnnnnntccccgcgtcgacggatc

SEQ ID NO: 5 - DNA, 58 bp, Artificial sequence
  Single strand DNA oligonucleotide
caagcagaagacggcatacgagatgtgactggagttcagacgtgtgctcttccgatct

SEQ ID NO: 6 - DNA, 19 bp, Artificial sequence
  Single strand DNA oligonucleotide
tccccgcgtcgacggatcc

SEQ ID NO: 7 - DNA, 39 bp, Artificial sequence
  Single strand DNA oligonucleotide
acacgacgctcttccgatctcctggtagcccaggtaggc

SEQ ID NO: 8 - DNA, 48 bp, Artificial sequence
  Single strand DNA oligonucleotide
ctggagttcagacgtgtgctcttccgatcttctccgacctcttcgccg

SEQ ID NO: 9 - DNA, 40 bp, Artificial sequence
  Single strand DNA oligonucleotide
acacgacgctcttccgatcttgtctggttaacagcctttg

SEQ ID NO: 10 - DNA, 50 bp, Artificial sequence
  Single strand DNA oligonucleotide
ctggagttcagacgtgtgctcttccgatctccatttcccatcctaacttc

SEQ ID NO: 11 - DNA, 58 bp, Artificial sequence
  Single strand DNA oligonucleotide
aatgatacggcgaccaccgagatctacactctttccctacacgacgctcttccgatct

SEQ ID NO: 12 - DNA, 55 bp, Artificial sequence
  Single strand DNA oligonucleotide
  misc_feature (25)..(31): n is a, c, g, or t
caagcagaagacggcatacgagatnnnnnnngtgactggagttcagacgtgtgct

SEQ ID NO: 13 - RNA, 6 nt, Artificial sequence
  polyadenylation signal sequence
aauaaa

SEQ ID NO: 14 - DNA, 35 bp, Artificial sequence
  T7 RNA polymerase promoter sequence
cgattgaggccggtaatacgactcactataggggc

SEQ ID NO: 15 - DNA, 8444 bp, Artificial sequence
  Sequences of exemplary constructs with BFP
atcccctgattctgtggataaccgtattaccgcctttgagtgagctgataccgctcgccgcagccgaacgaccgagcgcagcgagtcagtgagcgaggaagcggaagagcgcccaatacgcaaaccgcctctccccgcgcgttggccgattcattaatgcagctggcacgacaggtttcccgactggaaagcgggcagtgagcgcaacgcaattaatgtgagttagctcactcattaggcaccccaggctttacactttatgcttccggctcgtatgttgtgtggaattgtgagcggataacaatttcacacaggaaacagctatgaccatgattacgccaagcgcgcaattaaccctcactaaagggaacaaaagctggagctgcaagcttaatgtagtcttatgcaatactcttgtagtcttgcaacatggtaacgatgagttagcaacatgccttacaaggagagaaaaagcaccgtgcatgccgattggtggaagtaaggtggtacgatcgtgccttattaggaaggcaacagacgggtctgacatggattggacgaaccactgaattgccgcattgcagagatattgtatttaagtgcctagctcgatacataaacgggtctctctggttagaccagatctgagcctgggagctctctggctaactagggaacccactgcttaagcctcaataaagcttgccttgagtgcttcaagtagtgtgtgcccgtctgttgtgtgactctggtaactagagatccctcagacccttttagtcagtgtggaaaatctctagcagtggcgcccgaacagggacttgaaagcgaaagggaaaccagaggagctctctcgacgcaggactcggcttgctgaagcgcgcacggcaagaggcgaggggcggcgactggtgagtacgccaaaaattttgactagcggaggctagaaggagagagatgggtgcgagagcgtcagtattaagcgggggagaattagatcgcgatgggaaaaaattcggttaaggccagggggaaagaaaaaatataaattaaaacatatagtatgggcaagcagggagctagaacgattcgcagttaatcctggcctgttagaaacatcagaaggctgtagacaaatactgggacagctacaaccatcccttcagacaggatcagaagaacttagatcattatataatacagtagcaaccctctattgtgtgcatcaaaggatagagataaaagacaccaaggaagctttagacaagatagaggaagagcaaaacaaaagtaagaccaccgcacagcaagcggccgctgatcttcagacctggaggaggagatatgagggacaattggagaagtgaattatataaatataaagtagtaaaaattgaaccattaggagtagcacccaccaaggcaaagagaagagtggtgcagagagaaaaaagagcagtgggaataggagctttgttccttgggttcttgggagcagcaggaagcactatgggcgcagcgtcaatgacgctgacggtacaggccagacaattattgtctggtatagtgcagcagcagaacaatttgctgagggctattgaggcgcaacagcatctgttgcaactcacagtctggggcatcaagcagctccaggcaagaatcctggctgtggaaagatacctaaaggatcaacagctcctggggatttggggttgctctggaaaactcatttgcaccactgctgtgccttggaatgctagttggagtaataaatctctggaacagatttggaatcacacgacctggatggagtgggacagagaaattaacaattacacaagcttaatacactccttaattgaagaatcgcaaaaccagcaagaaaagaatgaacaagaattattggaattagataaatgggcaagtttgtggaattggtttaacataacaaattggctgtggtatataaaattattcataatgatagtaggaggcttggtaggtttaagaatagtttttgctgtactttctatagtgaatagagttaggcagggatattcaccattatcgtttcagacccacctcccaaccccgaggggacccagagagggcctatttcccatgattccttcatatttgcatatacgatacaaggctgttagagagataattagaattaatttgactgtaaacacaaagatattagtacaaaatacgtgacgtagaaagtaataatttcttgggtagtttgcagttttaaaattatgttttaaaatggactatcatatgcttaccgtaacttgaaagtatttcgatttcttggctttatatatcttgtggaaaggacgaaacaccggagacggacgtctctgttttagagctagaaatagcaagttaaaataaggctagtccgttatcaacttgaaaaagtggcaccgagtcggtgcttttttaagcttggcgtaactagatcttgagacaaatggcagtattcatccacaattttaaaagaaaaggggggattggggggtacagtgcaggggaaagaatagtagacataatagcaacagacatacaaactaaagaattacaaaaacaaattacaaaaattcaaaattttcgggtttattacagggacagcagagatccactttggcgccggctcgagggggcccgggtgcaaagatggataaagttttaaacagagaggaatctttgcagctaatggaccttctaggtcttgaaaggagtgggaattggctccggtgcccgtcagtgggcagagcgcacatcgcccacagtccccgagaagttggggggaggggtcggcaattgatccggtgcctagagaaggtggcgcggggtaaactgggaaagtgatgtcgtgtactggctccgcctttttcccgagggtgggggagaaccgtatataagtgcagtagtcgccgtgaacgttctttttcgcaacgggtttgccgccagaacacaggtaagtgccgtgtgtggttcccgcgggcctggcctctttacgggttatggcccttgcgtgccttgaattacttccactggctgcagtacgtgattcttgatcccgagcttcgggttggaagtgggtgggagagttcgaggccttgcgcttaaggagccccttcgcctcgtgcttgagttgaggcctggcctgggcgctggggccgccgcgtgcgaatctggtggcaccttcgcgcctgtctcgctgctttcgataagtctctagccatttaaaatttttgatgacctgctgcgacgctttttttctggcaagatagtcttgtaaatgcgggccaagatctgcacactggtatttcggtttttggggccgcgggcggcgacggggcccgtgcgtcccagcgcacatgttcggcgaggcggggcctgcgagcgcggccaccgagaatcggacgggggtagtctcaagctggccggcctgctctggtgcctggcctcgcgccgccgtgtatcgccccgccctgggcggcaaggctggcccggtcggcaccagttgcgtgagcggaaagatggccgcttcccggccctgctgcagggagctcaaaatggaggacgcggcgctcgggagagcgggcgggtgagtcacccacacaaaggaaaagggcctttccgtcctcagccgtcgcttcatgtgactccacggagtaccgggcgccgtccaggcacctcgattagttctcgagcttttggagtacgtcgtctttaggttggggggaggggttttatgcgatggagtttccccacactgagtgggtggagactgaagttaggccagcttggcacttgatgtaattctccttggaatttgccctttttgagtttggatcttggttcattctcaagcctcagacagtggttcaaagtttttttcttccatttcaggtgtcgtgacgtacggccaccatggtgagcaagggcgaggagctgttcaccggggtggtgcccatcctggtcgagctggacggcgacgtaaacggccacaagttcagcgtgaggggcgagggcgagggcgatgccaccaacggcaagctgaccctgaagttcatctgcaccaccggcaagctgcccgtgccctggcccaccctcgtgaccaccctgagccacggcgtgcagtgcttcgcccgctaccccgaccacatgaagcagcacgacttcttcaagtccgccatgcccgaaggctacgtccaggagcgcaccatcttcttcaaggacgacggcacctacaagacccgcgccgaggtgaagttcgagggcgacaccctggtgaaccgcatcgagctgaagggcgtcgacttcaaggaggacggcaacatcctggggcacaagctggagtacaacttcaacagccacaacatctatatcatggccgtcaagcagaagaacggcatcaaggtgaacttcaagatccgccacaacgtggaggacggcagcgtgcagctcgccgaccactaccagcagaacacccccatcggcgacggccccgtgctgctgcccgacagccactacctgagcacccagtccgtgctgagcaaagaccccaacgagaagcgcgatcacatggtcctgctggagttccgcaccgccgccgggatcactctcggcatggacgagctgtacaagtaaacgcgttaagtcgagtcgacaatcaacctctggattacaaaatttgtgaaagattgactggtattcttaactatgttgctccttttacgctatgtggatacgctgctttaatgcctttgtatcatgctattgcttcccgtatggctttcattttctcctccttgtataaatcctggttgctgtctctttatgaggagttgtggcccgttgtcaggcaacgtggcgtggtgtgcactgtgtttgctgacgcaacccccactggttggggcattgccaccacctgtcagctcctttccgggactttcgctttccccctccctattgccacggcggaactcatcgccgcctgccttgcccgctgctggacaggggctcggctgttgggcactgacaattccgtggtgttgtcggggaaatcatcgtcctttccttggctgctcgcctgtgttgccacctggattctgcgcgggacgtccttctgctacgtcccttcggccctcaatccagcggaccttccttcccgcggcctgctgccggctctgcggcctcttccgcgtcttcgccttcgccctcagacgagtcggatctccctttgggccgcctccccgcgtcgacggatccggtgatgggacttacaaggcagctgtagatcttagccactttttaaaagaaaaggggggactggaagggctaattcactcccaacgaagacaagatctgctttttgcttgtactgggtctctctggttagaccagatctgagcctgggagctctctggctaactagggaacccactgcttaagcctcaataaagcttgccttgagtgcttcaagtagtgtgtgcccgtctgttgtgtgactctggtaactagagatccctcagacccttttagtcagtgtggaaaatctctagcagtacgtatagtagttcatgtcatcttattattcagtatttataacttgcaaagaaatgaatatcagagagtgagaggaacttgtttattgcagcttataatggttacaaataaagcaatagcatcacaaatttcacaaataaagcatttttttcactgcattctagttgtggtttgtccaaactcatcaatgtatcttatcatgtctggctctagctatcccgcccctaactccgcccatcccgcccctaactccgcccagttccgcccattctccgccccatggctgactaattttttttatttatgcagaggccgaggccgcctcggcctctgagctattccagaagtagtgaggaggcttttttggaggcctagggacgtacccaattcgccctatagtgagtcgtattacgcgcgctcactggccgtcgttttacaacgtcgtgactgggaaaaccctggcgttacccaacttaatcgccttgcagcacatccccctttcgccagctggcgtaatagcgaagaggcccgcaccgatcgcccttcccaacagttgcgcagcctgaatggcgaatgggacgcgccctgtagcggcgcattaagcgcggcgggtgtggtggttacgcgcagcgtgaccgctacacttgccagcgccctagcgcccgctcctttcgctttcttcccttcctttctcgccacgttcgccggctttccccgtcaagctctaaatcgggggctccctttagggttccgatttagtgctttacggcacctcgaccccaaaaaacttgattagggtgatggttcacgtagtgggccatcgccctgatagacggtttttcgccctttgacgttggagtccacgttctttaatagtggactcttgttccaaactggaacaacactcaaccctatctcggtctattcttttgatttataagggattttgccgatttcggcctattggttaaaaaatgagctgatttaacaaaaatttaacgcgaattttaacaaaatattaacgcttacaatttaggtggcacttttcggggaaatgtgcgcggaacccctatttgtttatttttctaaatacattcaaatatgtatccgctcatgagacaataaccctgataaatgcttcaataatattgaaaaaggaagagtatgagtattcaacatttccgtgtcgcccttattcccttttttgcggcattttgccttcctgtttttgctcacccagaaacgctggtgaaagtaaaagatgctgaagatcagttgggtgcacgagtgggttacatcgaactggatctcaacagcggtaagatccttgagagttttcgccccgaagaacgttttccaatgatgagcacttttaaagttctgctatgtggcgcggtattatcccgtattgacgccgggcaagagcaactcggtcgccgcatacactattctcagaatgacttggttgagtactcaccagtcacagaaaagcatcttacggatggcatgacagtaagagaattatgcagtgctgccataaccatgagtgataacactgcggccaacttacttctgacaacgatcggaggaccgaaggagctaaccgcttttttgcacaacatgggggatcatgtaactcgccttgatcgttgggaaccggagctgaatgaagccataccaaacgacgagcgtgacaccacgatgcctgtagcaatggcaacaacgttgcgcaaactattaactggcgaactacttactctagcttcccggcaacaattaatagactggatggaggcggataaagttgcaggaccacttctgcgctcggcccttccggctggctggtttattgctgataaatctggagccggtgagcgtgggtctcgcggtatcattgcagcactggggccagatggtaagccctcccgtatcgtagttatctacacgacggggagtcaggcaactatggatgaacgaaatagacagatcgctgagataggtgcctcactgattaagcattggtaactgtcagaccaagtttactcatatatactttagattgatttaaaacttcatttttaatttaaaaggatctaggtgaagatcctttttgataatctcatgaccaaaatcccttaacgtgagttttcgttccactgagcgtcagaccccgtagaaaagatcaaaggatcttcttgagatcctttttttctgcgcgtaatctgctgcttgcaaacaaaaaaaccaccgctaccagcggtggtttgtttgccggatcaagagctaccaactctttttccgaaggtaactggcttcagcagagcgcagataccaaatactgttcttctagtgtagccgtagttaggccaccacttcaagaactctgtagcaccgcctacatacctcgctctgctaatcctgttaccagtggctgctgccagtggcgataagtcgtgtcttaccgggttggactcaagacgatagttaccggataaggcgcagcggtcgggctgaacggggggttcgtgcacacagcccagcttggagcgaacgacctacaccgaactgagatacctacagcgtgagctatgagaaagcgccacgcttcccgaagggagaaaggcggacaggtatccggtaagcggcagggtcggaacaggagagcgcacgagggagcttccagggggaaacgcctggtatctttatagtcctgtcgggtttcgccacctctgacttgagcgtcgatttttgtgatgctcgtcaggggggcggagcctatggaaaaacgccagcaacgcggcctttttacggttcctggccttttgctggccttttgctcacatgttctttcctgcgtt

SEQ ID NO: 16 - DNA, 8384 bp, Artificial sequence
  Sequences of exemplary constructs with BFP
atcccctgattctgtggataaccgtattaccgcctttgagtgagctgataccgctcgccgcagccgaacgaccgagcgcagcgagtcagtgagcgaggaagcggaagagcgcccaatacgcaaaccgcctctccccgcgcgttggccgattcattaatgcagctggcacgacaggtttcccgactggaaagcgggcagtgagcgcaacgcaattaatgtgagttagctcactcattaggcaccccaggctttacactttatgcttccggctcgtatgttgtgtggaattgtgagcggataacaatttcacacaggaaacagctatgaccatgattacgccaagcgcgcaattaaccctcactaaagggaacaaaagctggagctgcaagcttaatgtagtcttatgcaatactcttgtagtcttgcaacatggtaacgatgagttagcaacatgccttacaaggagagaaaaagcaccgtgcatgccgattggtggaagtaaggtggtacgatcgtgccttattaggaaggcaacagacgggtctgacatggattggacgaaccactgaattgccgcattgcagagatattgtatttaagtgcctagctcgatacataaacgggtctctctggttagaccagatctgagcctgggagctctctggctaactagggaacccactgcttaagcctcaataaagcttgccttgagtgcttcaagtagtgtgtgcccgtctgttgtgtgactctggtaactagagatccctcagacccttttagtcagtgtggaaaatctctagcagtggcgcccgaacagggacttgaaagcgaaagggaaaccagaggagctctctcgacgcaggactcggcttgctgaagcgcgcacggcaagaggcgaggggcggcgactggtgagtacgccaaaaattttgactagcggaggctagaaggagagagatgggtgcgagagcgtcagtattaagcgggggagaattagatcgcgatgggaaaaaattcggttaaggccagggggaaagaaaaaatataaattaaaacatatagtatgggcaagcagggagctagaacgattcgcagttaatcctggcctgttagaaacatcagaaggctgtagacaaatactgggacagctacaaccatcccttcagacaggatcagaagaacttagatcattatataatacagtagcaaccctctattgtgtgcatcaaaggatagagataaaagacaccaaggaagctttagacaagatagaggaagagcaaaacaaaagtaagaccaccgcacagcaagcggccgctgatcttcagacctggaggaggagatatgagggacaattggagaagtgaattatataaatataaagtagtaaaaattgaaccattaggagtagcacccaccaaggcaaagagaagagtggtgcagagagaaaaaagagcagtgggaataggagctttgttccttgggttcttgggagcagcaggaagcactatgggcgcagcgtcaatgacgctgacggtacaggccagacaattattgtctggtatagtgcagcagcagaacaatttgctgagggctattgaggcgcaacagcatctgttgcaactcacagtctggggcatcaagcagctccaggcaagaatcctggctgtggaaagatacctaaaggatcaacagctcctggggatttggggttgctctggaaaactcatttgcaccactgctgtgccttggaatgctagttggagtaataaatctctggaacagatttggaatcacacgacctggatggagtgggacagagaaattaacaattacacaagcttaatacactccttaattgaagaatcgcaaaaccagcaagaaaagaatgaacaagaattattggaattagataaatgggcaagtttgtggaattggtttaacataacaaattggctgtggtatataaaattattcataatgatagtaggaggcttggtaggtttaagaatagtttttgctgtactttctatagtgaatagagttaggcagggatattcaccattatcgtttcagacccacctcccaaccccgaggggacccagagagggcctatttcccatgattccttcatatttgcatatacgatacaaggctgttagagagataattagaattaatttgactgtaaacacaaagatattagtacaaaatacgtgacgtagaaagtaataatttcttgggtagtttgcagttttaaaattatgttttaaaatggactatcatatgcttaccgtaacttgaaagtatttcgatttcttggctttatatatcttgtggaaaggacgaaacaccggagacggacgtctctgttttagagctagaaatagcaagttaaaataaggctagtccgttatcaacttgaaaaagtggcaccgagtcggtgcttttttaagcttggcgtaactagatcttgagacaaatggcagtattcatccacaattttaaaagaaaaggggggattggggggtacagtgcaggggaaagaatagtagacataatagcaacagacatacaaactaaagaattacaaaaacaaattacaaaaattcaaaattttcgggtttattacagggacagcagagatccactttggcgccggctcgagggggcccgggtgcaaagatggataaagttttaaacagagaggaatctttgcagctaatggaccttctaggtcttgaaaggagtgggaattggctccggtgcccgtcagtgggcagagcgcacatcgcccacagtccccgagaagttggggggaggggtcggcaattgatccggtgcctagagaaggtggcgcggggtaaactgggaaagtgatgtcgtgtactggctccgcctttttcccgagggtgggggagaaccgtatataagtgcagtagtcgccgtgaacgttctttttcgcaacgggtttgccgccagaacacaggtaagtgccgtgtgtggttcccgcgggcctggcctctttacgggttatggcccttgcgtgccttgaattacttccactggctgcagtacgtgattcttgatcccgagcttcgggttggaagtgggtgggagagttcgaggccttgcgcttaaggagccccttcgcctcgtgcttgagttgaggcctggcctgggcgctggggccgccgcgtgcgaatctggtggcaccttcgcgcctgtctcgctgctttcgataagtctctagccatttaaaatttttgatgacctgctgcgacgctttttttctggcaagatagtcttgtaaatgcgggccaagatctgcacactggtatttcggtttttggggccgcgggcggcgacggggcccgtgcgtcccagcgcacatgttcggcgaggcggggcctgcgagcgcggccaccgagaatcggacgggggtagtctcaagctggccggcctgctctggtgcctggcctcgcgccgccgtgtatcgccccgccctgggcggcaaggctggcccggtcggcaccagttgcgtgagcggaaagatggccgcttcccggccctgctgcagggagctcaaaatggaggacgcggcgctcgggagagcgggcgggtgagtcacccacacaaaggaaaagggcctttccgtcctcagccgtcgcttcatgtgactccacggagtaccgggcgccgtccaggcacctcgattagttctcgagcttttggagtacgtcgtctttaggttggggggaggggttttatgcgatggagtttccccacactgagtgggtggagactgaagttaggccagcttggcacttgatgtaattctccttggaatttgccctttttgagtttggatcttggttcattctcaagcctcagacagtggttcaaagtttttttcttccatttcaggtgtcgtgacgtacggccaccatggtgagcaagggcgaggagctgttcaccggggtggtgcccatcctggtcgagctggacggcgacgtaaacggccacaagttcagcgtgaggggcgagggcgagggcgatgccaccaacggcaagctgaccctgaagttcatctgcaccaccggcaagctgcccgtgccctggcccaccctcgtgaccaccctgagccacggcgtgcagtgcttcgcccgctaccccgaccacatgaagcagcacgacttcttcaagtccgccatgcccgaaggctacgtccaggagcgcaccatcttcttcaaggacgacggcacctacaagacccgcgccgaggtgaagttcgagggcgacaccctggtgaaccgcatcgagctgaagggcgtcgacttcaaggaggacggcaacatcctggggcacaagctggagtacaacttcaacagccacaacatctatatcatggccgtcaagcagaagaacggcatcaaggtgaacttcaagatccgccacaacgtggaggacggcagcgtgcagctcgccgaccactaccagcagaacacccccatcggcgacggccccgtgctgctgcccgacagccactacctgagcacccagtccgtgctgagcaaagaccccaacgagaagcgcgatcacatggtcctgctggagttccgcaccgccgccgggatcactctcggcatggacgagctgtacaagtaaacgcgttaagtcgagtcgacaatcaacctctggattacaaaatttgtgaaagattgactggtattcttaactatgttgctccttttacgctatgtggatacgctgctttaatgcctttgtatcatgctattgcttcccgtatggctttcattttctcctccttgtataaatcctggttgctgtctctttatgaggagttgtggcccgttgtcaggcaacgtggcgtggtgtgcactgtgtttgctgacgcaacccccactggttggggcattgccaccacctgtcagctcctttccgggactttcgctttccccctccctattgccacggcggaactcatcgccgcctgccttgcccgctgctggacaggggctcggctgttgggcactgacaattccgtggtgttgtcggggaaatcatcgtcctttccttggctgctcgcctgtgttgccacctggattctgcgcgggacgtccttctgctacgtcccttcggccctcaatccagcggaccttccttcccgcggcctgctgccggctctgcggcctcttccgcgtcttcgccttcgccctcagacgagtcggatctccctttgggccgcctctccgcgtcgacggatccggtgatgggacttacaaggcagctgtagatcttagccactttttaaaagaaaaggggggactggaagggctaattcactcccaacgaagacaagatctgctttttgcttgtactgggtctctctggttagaccagatctgagcctgggagctctctggctaactagggaacccactgcttaagcctcaataaagcttgccttgagtgcttcaagtagtgtgtgcccgtctgttgtgtgactctggtaactagagatccctcagacccttttagtcagtgtggaaaatctctagcagtacgtatagtagttcatgtcatcttattattcagtatttataacttgcaaagaaatgaatatcagagagtgagaggaacttgtttattgcagcttataatggttacaaataaagcaatagcatcacaaatttcacaaataaagcatttttttcactgcattctagttgtggtttgtccaaactcatcaatgtatcttatcatgtctggctctagctatcccgcccctaactccgcccatcccgcccctaactccgcccagttccgcccattctccgccccatggctgactaattttttttatttatgcagaggccgaggccgcctcggcctctgagctattccagaagtagtgaggaggcttttttggaggcctagggacgtacccaattcgccctatagtgagtcgtattacgcgcgctcactggccgtcgttttacaacgtcgtgactgggaaaaccctggcgttacccaacttaatcgccttgcagcacatccccctttcgccagctggcgtaatagcgaagaggcccgcaccgatcgcccttcccaacagttgcgcagcctgaatggcgaatgggacgcgccctgtagcggcgcattaagcgcggcgggtgtggtggttacgcgcagcgtgaccgctacacttgccagcgccctagcgcccgctcctttcgctttcttcccttcctttctcgccacgttcgccggctttccccgtcaagctctaaatcgggggctccctttagggttccgatttagtgctttacggcacctcgaccccaaaaaacttgattagggtgatggttcacgtagtgggccatcgccctgatagacggtttttcgccctttgacgttggagtccacgttctttaatagtggactcttgttccaaactggaacaacactcaaccctatctcggtctattcttttgatttataagggattttgccgatttcggcctattggttaaaaaatgagctgatttaacaaaaatttaacgcgaattttaacaaaatattaacgcttacaatttaggtggcacttttcggggaaatgtgcgcggaacccctatttgtttatttttctaaatacattcaaatatgtatccgctcatgagacaataaccctgataaatgcttcaataatattgaaaaaggaagagtatgagtattcaacatttccgtgtcgcccttattcccttttttgcggcattttgccttcctgtttttgctcacccagaaacgctggtgaaagtaaaagatgctgaagatcagttgggtgcacgagtgggttacatcgaactggatctcaacagcggtaagatccttgagagttttcgccccgaagaacgttttccaatgatgagcacttttaaagttctgctatgtggcgcggtattatcccgtattgacgccgggcaagagcaactcggtcgccgcatacactattctcagaatgacttggttgagtactcaccagtcacagaaaagcatcttacggatggcatgacagtaagagaattatgcagtgctgccataaccatgagtgataacactgcggccaacttacttctgacaacgatcggaggaccgaaggagctaaccgcttttttgcacaacatgggggatcatgtaactcgccttgatcgttgggaaccggagctgaatgaagccataccaaacgacgagcgtgacaccacgatgcctgtagcaatggcaacaacgttgcgcaaactattaactggcgaactacttactctagcttcccggcaacaattaatagactggatggaggcggataaagttgcaggaccacttctgcgctcggcccttccggctggctggtttattgctgataaatctggagccggtgagcgtgggtctcgcggtatcattgcagcactggggccagatggtaagccctcccgtatcgtagttatctacacgacggggagtcaggcaactatggatgaacgaaatagacagatcgctgagataggtgcctcactgattaagcattggtaactgtcagaccaagtttactcatatatactttagattgatttaaaacttcatttttaatttaaaaggatctaggtgaagatcctttttgataatctcatgaccaaaatcccttaacgtgagttttcgttccactgagcgtcagaccccgtagaaaagatcaaaggatcttcttgagatcctttttttctgcgcgtaatctgctgcttgcaaacaaaaaaaccaccgctaccagcggtggtttgtttgccggatcaagagctaccaactctttttccgaaggtaactggcttcagcagagcgcagataccaaatactgttcttctagtgtagccgtagttaggccaccacttcaagaactctgtagcaccgcctacatacctcgctctgctaatcctgttaccagtggctgctgccagtggcgataagtcgtgtcttaccgggttggactcaagacgatagttaccggataaggcgcagcggtcgggctgaacggggggttcgtgcacacagcccagcttggagcgaacgacctacaccgaactgagatacctacagcgtgagctatgagaaagcgccacgcttcccgaagggagaaaggcggacaggtatccggtaagcggcagggtcggaacaggagagcgcacgagggagcttccagggggaaacgcctggtatctttatagtcctgtcgggtttcgccacctctgacttgagcgtcgatttttgtgatgctcgtcaggggggcggagcctatggaaaaacgccagcaacgc

SEQ ID NO: 17 - DNA, 8435 bp, Artificial sequence
  Sequences of exemplary constructs with  mcherry
cccgggtgcaaagatggataaagttttaaacagagaggaatctttgcagctaatggaccttctaggtcttgaaaggagtgggaattggctccggtgcccgtcagtgggcagagcgcacatcgcccacagtccccgagaagttggggggaggggtcggcaattgatccggtgcctagagaaggtggcgcggggtaaactgggaaagtgatgtcgtgtactggctccgcctttttcccgagggtgggggagaaccgtatataagtgcagtagtcgccgtgaacgttctttttcgcaacgggtttgccgccagaacacaggtaagtgccgtgtgtggttcccgcgggcctggcctctttacgggttatggcccttgcgtgccttgaattacttccactggctgcagtacgtgattcttgatcccgagcttcgggttggaagtgggtgggagagttcgaggccttgcgcttaaggagccccttcgcctcgtgcttgagttgaggcctggcctgggcgctggggccgccgcgtgcgaatctggtggcaccttcgcgcctgtctcgctgctttcgataagtctctagccatttaaaatttttgatgacctgctgcgacgctttttttctggcaagatagtcttgtaaatgcgggccaagatctgcacactggtatttcggtttttggggccgcgggcggcgacggggcccgtgcgtcccagcgcacatgttcggcgaggcggggcctgcgagcgcggccaccgagaatcggacgggggtagtctcaagctggccggcctgctctggtgcctggcctcgcgccgccgtgtatcgccccgccctgggcggcaaggctggcccggtcggcaccagttgcgtgagcggaaagatggccgcttcccggccctgctgcagggagctcaaaatggaggacgcggcgctcgggagagcgggcgggtgagtcacccacacaaaggaaaagggcctttccgtcctcagccgtcgcttcatgtgactccacggagtaccgggcgccgtccaggcacctcgattagttctcgagcttttggagtacgtcgtctttaggttggggggaggggttttatgcgatggagtttccccacactgagtgggtggagactgaagttaggccagcttggcacttgatgtaattctccttggaatttgccctttttgagtttggatcttggttcattctcaagcctcagacagtggttcaaagtttttttcttccatttcaggtgtcgtgacgtacggccaccatggtgagcaagggcgaggaggataacatggccatcatcaaggagttcatgcgcttcaaggtgcacatggagggctccgtgaacggccacgagttcgagatcgagggcgagggcgagggccgcccctacgagggcacccagaccgccaagctgaaggtgaccaagggtggccccctgcccttcgcctgggacatcctgtcccctcagttcatgtacggctccaaggcctacgtgaagcaccccgccgacatccccgactacttgaagctgtccttccccgagggcttcaagtgggagcgcgtgatgaacttcgaggacggcggcgtggtgaccgtgacccaggactcctccctgcaggacggcgagttcatctacaaggtgaagctgcgcggcaccaacttcccctccgacggccccgtaatgcagaagaagaccatgggctgggaggcctcctccgagcggatgtaccccgaggacggcgccctgaagggcgagatcaagcagaggctgaagctgaaggacggcggccactacgacgctgaggtcaagaccacctacaaggccaagaagcccgtgcagctgcccggcgcctacaacgtcaacatcaagttggacatcacctcccacaacgaggactacaccatcgtggaacagtacgaacgcgccgagggccgccactccaccggcggcatggacgagctgtacaagtaaacgcgttaagtcgagtcgacaatcaacctctggattacaaaatttgtgaaagattgactggtattcttaactatgttgctccttttacgctatgtggatacgctgctttaatgcctttgtatcatgctattgcttcccgtatggctttcattttctcctccttgtataaatcctggttgctgtctctttatgaggagttgtggcccgttgtcaggcaacgtggcgtggtgtgcactgtgtttgctgacgcaacccccactggttggggcattgccaccacctgtcagctcctttccgggactttcgctttccccctccctattgccacggcggaactcatcgccgcctgccttgcccgctgctggacaggggctcggctgttgggcactgacaattccgtggtgttgtcggggaaatcatcgtcctttccttggctgctcgcctgtgttgccacctggattctgcgcgggacgtccttctgctacgtcccttcggccctcaatccagcggaccttccttcccgcggcctgctgccggctctgcggcctcttccgcgtcttcgccttcgccctcagacgagtcggatctccctttgggccgcctccccgcgtcgacggatccggtgatgggacttacaaggcagctgtagatcttagccactttttaaaagaaaaggggggactggaagggctaattcactcccaacgaagacaagatctgctttttgcttgtactgggtctctctggttagaccagatctgagcctgggagctctctggctaactagggaacccactgcttaagcctcaataaagcttgccttgagtgcttcaagtagtgtgtgcccgtctgttgtgtgactctggtaactagagatccctcagacccttttagtcagtgtggaaaatctctagcagtacgtatagtagttcatgtcatcttattattcagtatttataacttgcaaagaaatgaatatcagagagtgagaggaacttgtttattgcagcttataatggttacaaataaagcaatagcatcacaaatttcacaaataaagcatttttttcactgcattctagttgtggtttgtccaaactcatcaatgtatcttatcatgtctggctctagctatcccgcccctaactccgcccatcccgcccctaactccgcccagttccgcccattctccgccccatggctgactaattttttttatttatgcagaggccgaggccgcctcggcctctgagctattccagaagtagtgaggaggcttttttggaggcctagggacgtacccaattcgccctatagtgagtcgtattacgcgcgctcactggccgtcgttttacaacgtcgtgactgggaaaaccctggcgttacccaacttaatcgccttgcagcacatccccctttcgccagctggcgtaatagcgaagaggcccgcaccgatcgcccttcccaacagttgcgcagcctgaatggcgaatgggacgcgccctgtagcggcgcattaagcgcggcgggtgtggtggttacgcgcagcgtgaccgctacacttgccagcgccctagcgcccgctcctttcgctttcttcccttcctttctcgccacgttcgccggctttccccgtcaagctctaaatcgggggctccctttagggttccgatttagtgctttacggcacctcgaccccaaaaaacttgattagggtgatggttcacgtagtgggccatcgccctgatagacggtttttcgccctttgacgttggagtccacgttctttaatagtggactcttgttccaaactggaacaacactcaaccctatctcggtctattcttttgatttataagggattttgccgatttcggcctattggttaaaaaatgagctgatttaacaaaaatttaacgcgaattttaacaaaatattaacgcttacaatttaggtggcacttttcggggaaatgtgcgcggaacccctatttgtttatttttctaaatacattcaaatatgtatccgctcatgagacaataaccctgataaatgcttcaataatattgaaaaaggaagagtatgagtattcaacatttccgtgtcgcccttattcccttttttgcggcattttgccttcctgtttttgctcacccagaaacgctggtgaaagtaaaagatgctgaagatcagttgggtgcacgagtgggttacatcgaactggatctcaacagcggtaagatccttgagagttttcgccccgaagaacgttttccaatgatgagcacttttaaagttctgctatgtggcgcggtattatcccgtattgacgccgggcaagagcaactcggtcgccgcatacactattctcagaatgacttggttgagtactcaccagtcacagaaaagcatcttacggatggcatgacagtaagagaattatgcagtgctgccataaccatgagtgataacactgcggccaacttacttctgacaacgatcggaggaccgaaggagctaaccgcttttttgcacaacatgggggatcatgtaactcgccttgatcgttgggaaccggagctgaatgaagccataccaaacgacgagcgtgacaccacgatgcctgtagcaatggcaacaacgttgcgcaaactattaactggcgaactacttactctagcttcccggcaacaattaatagactggatggaggcggataaagttgcaggaccacttctgcgctcggcccttccggctggctggtttattgctgataaatctggagccggtgagcgtgggtctcgcggtatcattgcagcactggggccagatggtaagccctcccgtatcgtagttatctacacgacggggagtcaggcaactatggatgaacgaaatagacagatcgctgagataggtgcctcactgattaagcattggtaactgtcagaccaagtttactcatatatactttagattgatttaaaacttcatttttaatttaaaaggatctaggtgaagatcctttttgataatctcatgaccaaaatcccttaacgtgagttttcgttccactgagcgtcagaccccgtagaaaagatcaaaggatcttcttgagatcctttttttctgcgcgtaatctgctgcttgcaaacaaaaaaaccaccgctaccagcggtggtttgtttgccggatcaagagctaccaactctttttccgaaggtaactggcttcagcagagcgcagataccaaatactgttcttctagtgtagccgtagttaggccaccacttcaagaactctgtagcaccgcctacatacctcgctctgctaatcctgttaccagtggctgctgccagtggcgataagtcgtgtcttaccgggttggactcaagacgatagttaccggataaggcgcagcggtcgggctgaacggggggttcgtgcacacagcccagcttggagcgaacgacctacaccgaactgagatacctacagcgtgagctatgagaaagcgccacgcttcccgaagggagaaaggcggacaggtatccggtaagcggcagggtcggaacaggagagcgcacgagggagcttccagggggaaacgcctggtatctttatagtcctgtcgggtttcgccacctctgacttgagcgtcgatttttgtgatgctcgtcaggggggcggagcctatggaaaaacgccagcaacgcggcctttttacggttcctggccttttgctggccttttgctcacatgttctttcctgcgttatcccctgattctgtggataaccgtattaccgcctttgagtgagctgataccgctcgccgcagccgaacgaccgagcgcagcgagtcagtgagcgaggaagcggaagagcgcccaatacgcaaaccgcctctccccgcgcgttggccgattcattaatgcagctggcacgacaggtttcccgactggaaagcgggcagtgagcgcaacgcaattaatgtgagttagctcactcattaggcaccccaggctttacactttatgcttccggctcgtatgttgtgtggaattgtgagcggataacaatttcacacaggaaacagctatgaccatgattacgccaagcgcgcaattaaccctcactaaagggaacaaaagctggagctgcaagcttaatgtagtcttatgcaatactcttgtagtcttgcaacatggtaacgatgagttagcaacatgccttacaaggagagaaaaagcaccgtgcatgccgattggtggaagtaaggtggtacgatcgtgccttattaggaaggcaacagacgggtctgacatggattggacgaaccactgaattgccgcattgcagagatattgtatttaagtgcctagctcgatacataaacgggtctctctggttagaccagatctgagcctgggagctctctggctaactagggaacccactgcttaagcctcaataaagcttgccttgagtgcttcaagtagtgtgtgcccgtctgttgtgtgactctggtaactagagatccctcagacccttttagtcagtgtggaaaatctctagcagtggcgcccgaacagggacttgaaagcgaaagggaaaccagaggagctctctcgacgcaggactcggcttgctgaagcgcgcacggcaagaggcgaggggcggcgactggtgagtacgccaaaaattttgactagcggaggctagaaggagagagatgggtgcgagagcgtcagtattaagcgggggagaattagatcgcgatgggaaaaaattcggttaaggccagggggaaagaaaaaatataaattaaaacatatagtatgggcaagcagggagctagaacgattcgcagttaatcctggcctgttagaaacatcagaaggctgtagacaaatactgggacagctacaaccatcccttcagacaggatcagaagaacttagatcattatataatacagtagcaaccctctattgtgtgcatcaaaggatagagataaaagacaccaaggaagctttagacaagatagaggaagagcaaaacaaaagtaagaccaccgcacagcaagcggccgctgatcttcagacctggaggaggagatatgagggacaattggagaagtgaattatataaatataaagtagtaaaaattgaaccattaggagtagcacccaccaaggcaaagagaagagtggtgcagagagaaaaaagagcagtgggaataggagctttgttccttgggttcttgggagcagcaggaagcactatgggcgcagcgtcaatgacgctgacggtacaggccagacaattattgtctggtatagtgcagcagcagaacaatttgctgagggctattgaggcgcaacagcatctgttgcaactcacagtctggggcatcaagcagctccaggcaagaatcctggctgtggaaagatacctaaaggatcaacagctcctggggatttggggttgctctggaaaactcatttgcaccactgctgtgccttggaatgctagttggagtaataaatctctggaacagatttggaatcacacgacctggatggagtgggacagagaaattaacaattacacaagcttaatacactccttaattgaagaatcgcaaaaccagcaagaaaagaatgaacaagaattattggaattagataaatgggcaagtttgtggaattggtttaacataacaaattggctgtggtatataaaattattcataatgatagtaggaggcttggtaggtttaagaatagtttttgctgtactttctatagtgaatagagttaggcagggatattcaccattatcgtttcagacccacctcccaaccccgaggggacccagagagggcctatttcccatgattccttcatatttgcatatacgatacaaggctgttagagagataattagaattaatttgactgtaaacacaaagatattagtacaaaatacgtgacgtagaaagtaataatttcttgggtagtttgcagttttaaaattatgttttaaaatggactatcatatgcttaccgtaacttgaaagtatttcgatttcttggctttatatatcttgtggaaaggacgaaacaccggagacggacgtctctgttttagagctagaaatagcaagttaaaataaggctagtccgttatcaacttgaaaaagtggcaccgagtcggtgcttttttaagcttggcgtaactagatcttgagacaaatggcagtattcatccacaattttaaaagaaaaggggggattggggggtacagtgcaggggaaagaatagtagacataatagcaacagacatacaaactaaagaattacaaaaacaaattacaaaaattcaaaattttcgggtttattacagggacagcagagatccactttggcgccggctcgaggggg